European Patent Application EP 4 442 806 A1, published October 9, 2024. Title: 一种抗氧化、减脂和抑制肿瘤生长的广西阿克曼氏菌及其产品与应用. Applicant: 广西爱生生命科技有限公司. The sequence listing filed with the application follows.

SEQUENCE LISTING (6 sequences)

SEQ ID NO: 1 - DNA, 20 bp, synthetic construct
  source 1..20: mol_type = other DNA
cagcacgtgaaggtggggac

SEQ ID NO: 2 - DNA, 20 bp, synthetic construct
  source 1..20: mol_type = other DNA
cagcacgtgaaggtggggac

SEQ ID NO: 3 - DNA, 20 bp, synthetic construct
  source 1..20: mol_type = other DNA
agagtttgatcctggctcag

SEQ ID NO: 4 - DNA, 22 bp, synthetic construct
  source 1..22: mol_type = other DNA
tacggctaccttgttacgactt

SEQ ID NO: 5 - DNA, 1400 bp, Akkermansia sp.
  source 1..1400: mol_type = genomic DNA
gcgggcgggtggaagacatgcaagtcgaacggaagaatgctagcttgctaatattcttcagtggcgcacgggtgagtaacacgtgagcaacctaccttcgagtgggggatagccccgggaaactgggattaataccgcatgaggtcgaaagatcaaagcagcaatgcgcttgaagatgggctcgcgtcctattagttagttggtgaggtaacggctcaccaaggcgatgacgggtagccggtctgagaggatgtccggccacactggaactgagacacggtccagacacctacgggtggcagcagtcgagaatcattcacaatgggggcaaccctgatggtgcgacgccgcgtgggggaagaaggtcttcggattgtaaacccctgtcatgtgggagcaagcagcaatgttgatagtaccacaagaggaagagacggctaactctgtgccagcagccgcggtaatacagaggtctcaagcgttgttcggaatcactgggcgtaaagagtacgtaggctgttttctaagtcaggtgtgaaaggcaggggctcaacccctggactgcacatgatactgggagactggagtaatggagggggaaccggaattctcggtgtagcagtgaaatgcgtagatatcgagaggaacactcgtggcgaaggcgggttcctggacattaactgacgctgaggtacgaaggccagggtagcgaaagggattagatacccctgtagtcctggcagtaaacggtgcacgcttggtgtgaggggactcgacccccctcgtgccggagctaacgcgttaagcgtgccgcctggggagtacggtcgcaagattaaaactcaaagaaattgacggggacccgcacaagcggtggagtatgtggcttaattcgatgcaacgcgaagaaccttacctgggcttgacatgtaatgaacaacatgtgaaagcatgcgactcttcggaggcgttacacaggtgctgcatggccgtcgtcagctcgtgtcgtgagatgtttggttaagtccagcaacgagcgcaacccctgtggccagttaccagcacgttatggtggggactctggcaagactgcccagatcaactgggaggaaggtggggacgacgtcaggtcagtatggcccttatgcccagggctgcacacgtactacaatgcccagaacagagggggccgaagccgtgaggcggaggaaatcctgaaaactgggcccagttcggactgtaggctgcaacccgcctacacgaagccggaatcgctagtaatggcgcatcagctacggcgccgtgaatacgttcccgggtcttgtacacaccgcccgtcacatcatggaagccggtcgcacccgaagtatctagagccaaccgcaaggaggcagggtccc

SEQ ID NO: 6 - DNA, 1409 bp, Akkermansia sp.
  source 1..1409: mol_type = genomic DNA
gcggggcgcgtgcaaaagacatgcaagtcgaacggaagaatgctagcttgctaatattcttcagtggcgcacgggtgagtaacacgtgagcaacctaccttcgagtgggggatagccccgggaaactgggattaataccgcatgaggtcgaaagatcaaagcagcaatgcgcttgaagatgggctcgcgtcctattagttagttggtgaggtaacggctcaccaaggcgatgacgggtagccggtctgagaggatgtccggccacactggaactgagacacggtccagacacctacgggtggcagcagtcgagaatcattcacaatgggggcaaccctgatggtgcgacgccgcgtgggggaagaaggtcttcggattgtaaacccctgtcatgtgggagcaagcagcaatgttgatagtaccacaagaggaagagacggctaactctgtgccagcagccgcggtaatacagaggtctcaagcgttgttcggaatcactgggcgtaaagagtacgtaggctgttttctaagtcaggtgtgaaaggcaggggctcaacccctggactgcacatgatactgggagactggagtaatggagggggaaccggaattctcggtgtagcagtgaaatgcgtagatatcgagaggaacactcgtggcgaaggcgggttcctggacattaactgacgctgaggtacgaaggccagggtagcgaaagggattagatacccctgtagtcctggcagtaaacggtgcacgcttggtgtgaggggactcgacccccctcgtgccggagctaacgcgttaagcgtgccgcctggggagtacggtcgcaagattaaaactcaaagaaattgacggggacccgcacaagcggtggagtatgtggcttaattcgatgcaacgcgaagaaccttacctgggcttgacatgtaatgaacaacatgtgaaagcatgcgactcttcggaggcgttacacaggtgctgcatggccgtcgtcagctcgtgtcgtgagatgtttggttaagtccagcaacgagcgcaacccctgtggccagttaccagcacgttatggtggggactctggcaagactgcccagatcaactgggaggaaggtggggacgacgtcaggtcagtatggcccttatgcccagggctgcacacgtactacaatgcccagaacagagggggccgaagccgtgaggcggaggaaatcctgaaaactgggcccagttcggactgtaggctgcaacccgcctacacgaagccggaatcgctagtaatggcgcatcagctacggcgccgtgaatacgttcccgggtcttgtacacaccgcccgtcacatcatggaagccggtcgcacccgaagtatctagagccaaccgcaaggaggcagggtcctaagggt